European Patent Application EP 4 438 623 A1, published October 2, 2024. Title: Novel Engineered Anti-spike IgG3 Antibodies. Applicant: Tanea Medical AB. The sequence listing filed with the application follows.

SEQUENCE LISTING (25 sequences)

SEQ ID NO: 1 - protein, 377 aa, synthetic construct
ASTKGPSVFPLAPCSRSTSGGTAALGCLVKDYFPEPVTVSWNSGALTSGVHTFPAVLQSSGLYSLSSVVTVPSSSLGTQTYTCNVNHKPSNTKVDKRVELKTPLGDTTHTCPRCPEPKSCDTPPPCPRCPEPKSCDTPPPCPRCPEPKSCDTPPPCPRCPAPELLGGPSVFLFPPKPKDTLMISRTPEVTCVVVDVSHEDPEVQFKWYVDGVEVHNAKTKPREEQFNSTFRVVSVLTVLHQDWLNGKEYKCKVSNKALPAPIEKTISKTKGQPREPQVYTLPPSREEMTKNQVSLTCLVKGFYPSDIAVEWESSGQPENNYNTTPPMLDSDGSFFLYSKLTVDKSRWQQGNIFSCSVMHEALHNRFTQKSLSLSPGK

SEQ ID NO: 2 - protein, 377 aa, synthetic construct
ASTKGPSVFPLAPCSRSTSGGTAALGCLVKDYFPEPVTVSWNSGALTSGVHTFPAVLQSSGLYSLSSVVTVPSSSLGTQTYTCNVNHKPSNTKVDKRVELKTPLGDTTHTCPRCPEPKSCDTPPPCPRCPEPKSCDTPPPCPRCPEPKSCDTPPPCPRCPAPELLGGPSVFLFPPKPKDTLMISRTPEVTCVVVDVSHEDPEVQFKWYVDGVEVHNAKTKPREEQFNSTFRVVSVLTVLHQDWLNGKEYKCKVSNKALPAPIEKTISKTKGQPREPQVYTLPPSREEMTKNQVSLTCLVKGFYPSDIAVEWESSGQPENNYKTTPPVLDSDGSFFLYSKLTVDKSRWQQGNIFSCSVMHEALHNHFTQKSLSLSPGK

SEQ ID NO: 3 - protein, 377 aa, synthetic construct
ASTKGPSVFPLAPSSKSTSGGTAALGCLVKDYFPEPVTVSWNSGALTSGVHTFPAVLQSSGLYSLSSVVTVPSSSLGTQTYICNVNHKPSNTKVDKKVELKTPLGDTTHTCPRCPEPKSCDTPPPCPRCPEPKSCDTPPPCPRCPEPKSCDTPPPCPRCPAPELLGGPSVFLFPPKPKDTLMISRTPEVTCVVVDVSHEDPEVKFNWYVDGVEVHNAKTKPREEQYNSTYRVVSVLTVLHQDWLNGKEYKCKVSNKALPAPIEKTISKAKGQPREPQVYTLPPSRDELTKNQVSLTCLVKGFYPSDIAVEWESNGQPENNYKTTPPVLDSDGSFFLYSKLTVDKSRWQQGNVFSCSVMHEALHNHYTQKSLSLSPGK

SEQ ID NO: 4 - protein, 1270 aa, synthetic construct
MFVFLVLLPLVSSQCVNLTTRTQLPPAYTNSFTRGVYYPDKVFRSSVLHSTQDLFLPFFSNVTWFHAISGTNGTKRFDNPVLPFNDGVYFASTEKSNIIRGWIFGTTLDSKTQSLLIVNNATNVVIKVCEFQFCNDPFLGVYHKNNKSWMESEFRVYSSANNCTFEYVSQPFLMDLEGKQGNFKNLREFVFKNIDGYFKIYSKHTPINLVRDLPQGFSALEPLVDLPIGINITRFQTLLALHRSYLTPGDSSSGWTAGAAAYYVGYLQPRTFLLKYNENGTITDAVDCALDPLSETKCTLKSFTVEKGIYQTSNFRVQPTESIVRFPNITNLCPFGEVFNATRFASVYAWNRKRISNCVADYSVLYNSASFSTFKCYGVSPTKLNDLCFTNVYADSFVIRGDEVRQIAPGQTGKIADYNYKLPDDFTGCVIAWNSNNLDSKVGGNYNYLYRLFRKSNLKPFERDISTEIYQAGSTPCNGVEGFNCYFPLQSYGFQPTYGVGYQPYRVVVLSFELLHAPATVCGPKKSTNLVKNKCVNFNFNGLTGTGVLTESNKKFLPFQQFGRDIDDTTDAVRDPQTLEILDITPCSFGGVSVITPGTNTSNQVAVLYQGVNCTEVPVAIHADQLTPTWRVYSTGSNVFQTRAGCLIGAEHVNNSYECDIPIGAGICASYQTQTNSHRRARSVASQSIIAYTMSLGAENSVAYSNNSIAIPINFTISVTTEILPVSMTKTSVDCTMYICGDSTECSNLLLQYGSFCTQLNRALTGIAVEQDKNTQEVFAQVKQIYKTPPIKDFGGFNFSQILPDPSKPSKRSFIEDLLFNKVTLADAGFIKQYGDCLGDIAARDLICAQKFNGLTVLPPLLTDEMIAQYTSALLAGTITSGWTFGAGAALQIPFAMQMAYRFNGIGVTQNVLYENQKLIANQFNSAIGKIQDSLSSTASALGKLQDVVNQNAQALNTLVKQLSSNFGAISSVLNDILARLDKVEAEVQIDRLITGRLQSLQTYVTQQLIRAAEIRASANLAATKMSECVLGQSKRVDFCGKGYHLMSFPQSAPHGVVFLHVTYVPAQEKNFTTAPAICHDGKAHFPREGVFVSNGTHWFVTQRNFYEPQIITTHNTFVSGNCDVVIGIVNNTVYDPLQPELDSFKEELDKYFKNHTSPDVDLGDISGINASVVNIQKEIDRLNEVAKNLNESLIDLQELGKYEQYIKWPWYIWLGFIAGLIAIVMVTIMLCCMTSCCSCLKGCCSCGSCCKFDEDDSEPVLKGVKLHYT

SEQ ID NO: 5 - protein, 1271 aa, synthetic construct
MFVFLVLLPLVSSQCVNLRTRTQLPPAYTNSFTRGVYYPDKVFRSSVLHSTQDLFLPFFSNVTWFHAIHVSGTNGTTRFDNPVLPFNDGVYFASTEKSNIIRGWIFGTTLDSKTQSLLIVNNATNVVIKVCEFQFCNDPFLGVYYHKNNKSWMESGVYSSANNCTFEYVSQPFLMDLEGKQGNFKNLREFVFKNIDGYFKIYSKHTPINLVRDLPQGFSALEPLVDLPIGINITRFQTLLALHRSYLTPGDSSSGWTAGAAAYYVGYLQPRTFLLKYNENGTITDAVDCALDPLSETKCTLKSFTVEKGIYQTSNFRVQPTESIVRFPNITNLCPFGEVFNATRFASVYAWNRKRISNCVADYSVLYNSASFSTFKCYGVSPTKLNDLCFTNVYADSFVIRGDEVRQIAPGQTGKIADYNYKLPDDFTGCVIAWNSNNLDSKVGGNYNYRYRLFRKSNLKPFERDISTEIYQAGSKPCNGVEGFNCYFPLQSYGFQPTNGVGYQPYRVVVLSFELLHAPATVCGPKKSTNLVKNKCVNFNFNGLTGTGVLTESNKKFLPFQQFGRDIADTTDAVRDPQTLEILDITPCSFGGVSVITPGTNTSNQVAVLYQGVNCTEVPVAIHADQLTPTWRVYSTGSNVFQTRAGCLIGAEHVNNSYECDIPIGAGICASYQTQTNSRRRARSVASQSIIAYTMSLGAENSVAYSNNSIAIPTNFTISVTTEILPVSMTKTSVDCTMYICGDSTECSNLLLQYGSFCTQLNRALTGIAVEQDKNTQEVFAQVKQIYKTPPIKDFGGFNFSQILPDPSKPSKRSFIEDLLFNKVTLADAGFIKQYGDCLGDIAARDLICAQKFNGLTVLPPLLTDEMIAQYTSALLAGTITSGWTFGAGAALQIPFAMQMAYRFNGIGVTQNVLYENQKLIANQFNSAIGKIQDSLSSTASALGKLQNVVNQNAQALNTLVKQLSSNFGAISSVLNDILSRLDKVEAEVQIDRLITGRLQSLQTYVTQQLIRAAEIRASANLAATKMSECVLGQSKRVDFCGKGYHLMSFPQSAPHGVVFLHVTYVPAQEKNFTTAPAICHDGKAHFPREGVFVSNGTHWFVTQRNFYEPQIITTDNTFVSGNCDVVIGIVNNTVYDPLQPELDSFKEELDKYFKNHTSPDVDLGDISGINASVVNIQKEIDRLNEVAKNLNESLIDLQELGKYEQYIKWPWYIWLGFIAGLIAIVMVTIMLCCMTSCCSCLKGCCSCGSCCKFDEDDSEPVLKGVKLHYT

SEQ ID NO: 6 - protein, 1270 aa, synthetic construct
MFVFLVLLPLVSSQCVNLTTRTQLPPAYTNSFTRGVYYPDKVFRSSVLHSTQDLFLPFFSNVTWFHVISGTNGTKRFDNPVLPFNDGVYFASIEKSNIIRGWIFGTTLDSKTQSLLIVNNATNVVIKVCEFQFCNDPFLDHKNNKSWMESEFRVYSSANNCTFEYVSQPFLMDLEGKQGNFKNLREFVFKNIDGYFKIYSKHTPIIVREPEDLPQGFSALEPLVDLPIGINITRFQTLLALHRSYLTPGDSSSGWTAGAAAYYVGYLQPRTFLLKYNENGTITDAVDCALDPLSETKCTLKSFTVEKGIYQTSNFRVQPTESIVRFPNITNLCPFDEVFNATRFASVYAWNRKRISNCVADYSVLYNLAPFFTFKCYGVSPTKLNDLCFTNVYADSFVIRGDEVRQIAPGQTGNIADYNYKLPDDFTGCVIAWNSNKLDSKVSGNYNYLYRLFRKSNLKPFERDISTEIYQAGNKPCNGVAGFNCYFPLRSYSFRPTYGVGHQPYRVVVLSFELLHAPATVCGPKKSTNLVKNKCVNFNFNGLKGTGVLTESNKKFLPFQQFGRDIADTTDAVRDPQTLEILDITPCSFGGVSVITPGTNTSNQVAVLYQGVNCTEVPVAIHADQLTPTWRVYSTGSNVFQTRAGCLIGAEYVNNSYECDIPIGAGICASYQTQTKSHRRARSVASQSIIAYTMSLGAENSVAYSNNSIAIPTNFTISVTTEILPVSMTKTSVDCTMYICGDSTECSNLLLQYGSFCTQLKRALTGIAVEQDKNTQEVFAQVKQIYKTPPIKYFGGFNFSQILPDPSKPSKRSFIEDLLFNKVTLADAGFIKQYGDCLGDIAARDLICAQKFKGLTVLPPLLTDEMIAQYTSALLAGTITSGWTFGAGAALQIPFAMQMAYRFNGIGVTQNVLYENQKLIANQFNSAIGKIQDSLSSTASALGKLQDVVNHNAQALNTLVKQLSSKFGAISSVLNDIFSRLDKVEAEVQIDRLITGRLQSLQTYVTQQLIRAAEIRASANLAATKMSECVLGQSKRVDFCGKGYHLMSFPQSAPHGVVFLHVTYVPAQEKNFTTAPAICHDGKAHFPREGVFVSNGTHWFVTQRNFYEPQIITTDNTFVSGNCDVVIGIVNNTVYDPLQPELDSFKEELDKYFKNHTSPDVDLGDISGINASVVNIQKEIDRLNEVAKNLNESLIDLQELGKYEQYIKWPWYIWLGFIAGLIAIVMVTIMLCCMTSCCSCLKGCCSCGSCCKFDEDDSEPVLKGVKLHYT

SEQ ID NO: 7 - protein, 62 aa, Homo sapiens
ELKTPLGDTTHTCPRCPEPKSCDTPPPCPRCPEPKSCDTPPPCPRCPEPKSCDTPPPCPRCP

SEQ ID NO: 8 - protein, 17 aa, synthetic construct
ELKTPLGDTTHTCPRCP

SEQ ID NO: 9 - protein, 15 aa, synthetic construct
EPSKCDTPPPCPRCP

SEQ ID NO: 10 - protein, 121 aa, synthetic construct
QVTLKESGPVLVKPTETLTLTCTVSGFSLSNAKMGVSWIRQPPGKALEWLAHIFSNDEKSYSTSLKSSLTISKDTSKSQVVLTMTNMDPVDTATYYCARLLWFGGNYFDYWGQGTLVTVSS

SEQ ID NO: 11 - protein, 105 aa, synthetic construct
SYELTQPLSVSVALGQTARITCGGNNIGSKMHWYQQKPGQAPVLVIYRDSNRPSGIPERFSGSNSGNTATLTISRAQAGDEADYYCQVWDSSTVVFGGGTKLTVL

SEQ ID NO: 12 - protein, 126 aa, synthetic construct
QVQLVQSGAEVKKPGASVKVSCKASGYTFTSHAVHWVRQAPGQRLEWMGWINAGNGNTKYSQKFQGRVTITRDTSASTAYMELSSLRSEDTAVYYCARDPVLRYFDWTTPYYFDYWGQGTLVTVSS

SEQ ID NO: 13 - protein, 108 aa, synthetic construct
EIVLTQSPGTLSLSPGERATLSCRASQSFSSSYLAWYQQKPGQAPRLLIYGASSRATGIPDRFSGSGSGTDFTLTISRLEPEDFAVYYCQHYGSSPLTFGGGTKVEIK

SEQ ID NO: 14 - protein, 119 aa, synthetic construct
QVTLRESGPALVRPTQTLTLTCTFSGFSLSTSGMCVSWIRQPPGKALEWLARIDWDDDKYYSTSLRTRLTISKDTSKNQVVLTMTNMDPVDTATYYCARMTVTTAFDIWGQGTMVTVSS

SEQ ID NO: 15 - protein, 107 aa, synthetic construct
DIQMTQSPSSLSASVGDRVTITCRASQSISSYLNWYQQKPGKAPKLLIYAASSLQSGVPSRFSGSGSGTDFTLTISSLQPEDFATYYCQQSYSTPRTFGQGTKVEIK

SEQ ID NO: 16 - protein, 127 aa, synthetic construct
QVQLVQSGAEVKKPGASVKVSCKASGYTFTSYDINWVRQATGQGLEWMGWMNPNSGNTAYAQKFQGRVTMTRNTSISTAYMELSSLRSEDTAVYYCARGGRYCSSTSCYSGVPNDYWGQGTLVTVSS

SEQ ID NO: 17 - protein, 107 aa, synthetic construct
DIQLTQSPSFLSASVGDRVTITCRASQGVSSYLAWYQQKPGKAPKLLIYPASTLQSGVPSRFSGSGSGTEFTLTISSLQPEDFATYYCQQLNSYPLTFGGGTKVEIK

SEQ ID NO: 18 - protein, 128 aa, synthetic construct
EVQLVESGGGLVKPGGSLRLSCAASGFTFSSYSMNWVRQAPGKGLEWVSSISSSSSYIYYADSVKGRFTISRDNAKNSLYLQMNSLRAEDTAVYYCARRSFVSSSTDDYYYYYDMDVWGQGTTVTVSS

SEQ ID NO: 19 - protein, 108 aa, synthetic construct
SYELTQPPSVSVSPGQTARITCSGDALPKQYAYWYQQKPGQAPVLVIYKDSERPSGIPERFSGSSSGTTVTLTISGVQAEDEADYYCQSADSSGTYVVFAGGTKLTVL

SEQ ID NO: 20 - protein, 123 aa, synthetic construct
QVQLVESGGGVVQPGRSLRLSCAASGFTFSSYDMHWVRQAPGKGLEWVALISYDGSNTYYADSVKGRFTISRDNSKNTLYLQMNSLRAEDTAVFYCAKTIYSYALKPNYFDYWGQGTLVTVSS

SEQ ID NO: 21 - protein, 107 aa, synthetic construct
DIQMTQSPSSLSASVGDRVTITCQASQDISNYLNWYQQKPGKAPKLLIYDASNLETGVPSRFSGSGSGTDFTFTISSLQPEDIATYYCQQYDNLPPTFGGGTKVGIK

SEQ ID NO: 22 - protein, 121 aa, synthetic construct
QVQLVQSGAEVKKPGASVKVSCKASGYTFTSYGISWVRQAPGQGLEWMGWISAYNGNTNYAQKVQGRVTMTRDTSTSTAYMELRSLRSDDTAVYYCARDGIAVAEDWFDPWGQGTLVTVSS

SEQ ID NO: 23 - protein, 108 aa, synthetic construct
SYELTQPPSVSVAPGKTARITCGENNIGSKSVHWYQQKPGQAPVLVIYYDSDRPSGIPERFSGSNSGNTATLTISRVEAGDEADYYCQVWDGSSDHVVFGGGTKLTVL

SEQ ID NO: 24 - protein, 120 aa, synthetic construct
QVQLQESGPRLVKPSGTLSLTCAVSGGSISSSNWWTWVRQPPGKGLEWIGEIYHSGSTNYTPSLKSRVTISVDKSKNQFSLRLNSVTAADTAVYYCARGWSSSWYGLDYWGQGTLVTVSS

SEQ ID NO: 25 - protein, 110 aa, synthetic construct
QSALTQPASVSGSPGQSITISCTGTSSDVGSYNLVSWYQQHPGKAPKLVIYEATKRPSGVSNRFSGSKSGNTASLTISGLQAEDEADYYCYSYAGSSTWVFGGGTKLTVL